European Patent Application EP 4 371 556 A1, published May 22, 2024. Title: Angiotensin(1-7) pharmaceutical compositions for inhalation. Applicant: Explicat Pharma GmbH. The sequence listing filed with the application follows.

SEQUENCE LISTING (16 sequences)

SEQ ID NO: 1 - protein, 8 aa, Homo sapiens
DRVYIHPF

SEQ ID NO: 2 - protein, 7 aa, Homo sapiens
DRVYIHP

SEQ ID NO: 3 - protein, 10 aa, Homo sapiens
DRVYIHPFHL

SEQ ID NO: 4 - protein, 5 aa, Homo sapiens
DRVYI

SEQ ID NO: 5 - protein, 7 aa, synthetic construct
  SITE 1: note = sarcosine
XRVYIHP

SEQ ID NO: 6 - protein, 7 aa, synthetic construct
  SITE 7: note = D-alanine
DRVYIHX

SEQ ID NO: 7 - protein, 7 aa, synthetic construct
  SITE 7: note = D-proline
DRVYIHX

SEQ ID NO: 8 - protein, 7 aa, synthetic construct
ARVYIHP

SEQ ID NO: 9 - protein, 7 aa, synthetic construct
DRVAIHP

SEQ ID NO: 10 - protein, 7 aa, synthetic construct
DRPYIHP

SEQ ID NO: 11 - protein, 7 aa, synthetic construct
DRKYIHP

SEQ ID NO: 12 - protein, 7 aa, synthetic construct
  SITE 3: note = norLeucine
DRXYIHP

SEQ ID NO: 13 - protein, 7 aa, synthetic construct
DRPAIHP

SEQ ID NO: 14 - protein, 7 aa, synthetic construct
  SITE 3: note = 3Hyp
DRXYIHP

SEQ ID NO: 15 - protein, 7 aa, synthetic construct
  SITE 3: note = 4Hyp
DRXYIHP

SEQ ID NO: 16 - protein, 8 aa, synthetic construct
RDRVYIHP